European Patent Specification EP 3 684 799 B1, published July 8, 2026. Title: HLA CLASS II-RESTRICTED T CELL RECEPTORS AGAINST MUTATED RAS. Applicant: THE UNITED STATES OF AMERICA, AS REPRESENTED BY THE SECRETARY, DEPARTMENT OF HEALTH AND HUMAN SERVICES. The sequence listing filed with the application follows.

SEQUENCE LISTING (56 sequences)

SEQ ID NO: 1 - protein, 6 aa, Homo sapiens
DSASNY

SEQ ID NO: 2 - protein, 7 aa, Homo sapiens
IRSNVGE

SEQ ID NO: 3 - protein, 13 aa, Homo sapiens
CAASTGGGNKLTF

SEQ ID NO: 4 - protein, 6 aa, Homo sapiens
DFQATT

SEQ ID NO: 5 - protein, 7 aa, Homo sapiens
SNEGSKA

SEQ ID NO: 6 - protein, 15 aa, Homo sapiens
CSAREGAGGMGTQYF

SEQ ID NO: 7 - protein, 6 aa, Homo sapiens
SSNFYA

SEQ ID NO: 8 - protein, 7 aa, Homo sapiens
MTLNGDE

SEQ ID NO: 9 - protein, 11 aa, Homo sapiens
CAFTTGNQFYF

SEQ ID NO: 10 - protein, 6 aa, Homo sapiens
SGHDYL

SEQ ID NO: 11 - protein, 6 aa, Homo sapiens
FNNNVP

SEQ ID NO: 12 - protein, 16 aa, Homo sapiens
CASSSYGGYSNQPQHF

SEQ ID NO: 13 - protein, 131 aa, Homo sapiens
MTSIRAVFIFLWLQLDLVNGENVEQHPSTLSVQEGDSAVIKCTYSDSASNYFPWYKQELGKGPQLIIDIRSNVGEKKDQRIAVTLNKTAKHFSLHITETQPEDSAVYFCAASTGGGNKLTFGTGTQLKVEL

SEQ ID NO: 14 - protein, 132 aa, Homo sapiens
MLLLLLLLGPAGSGLGAVVSQHPSRVICKSGTSVKIECRSLDFQATTMFWYRQFPKQSLMLMATSNEGSKATYEQGVEKDKFLINHASLTLSTLTVTSAHPEDSSFYICSAREGAGGMGTQYFGPGTRLLVL

SEQ ID NO: 15 - protein, 132 aa, Homo sapiens
MEKNPLAAPLLILWFHLDCVSSILNVEQSPQSLHVQEGDSTNFTCSFPSSNFYALHWYRWETAKSPEALFVMTLNGDEKKKGRISATLNTKEGYSYLYIKGSQPEDSATYLCAFTTGNQFYFGTGTSLTVIP

SEQ ID NO: 16 - protein, 137 aa, Homo sapiens
MGSWTLCCVSLCILVAKHTDAGVIQSPRHEVTEMGQEVTLRCKPISGHDYLFWYRQTMMRGLELLIYFNNNVPIDDSGMPEDRFSAKMPNASFSTLKIQPSEPRDSAVYFCASSSYGGYSNQPQHFGDGTRLSILED

SEQ ID NO: 17 - protein, 189 aa, Homo sapiens [sequence omitted]

SEQ ID NO: 18 - protein, 188 aa, Homo sapiens [sequence omitted]

SEQ ID NO: 19 - protein, 189 aa, Homo sapiens
MTEYKLVVVGAGGVGKSALTIQLIQNHFVDEYDPTIEDSYRKQVVIDGETCLLDILDTAGQEEYSAMRDQYMRTGEGFLCVFAINNTKSFEDIHQYREQIKRVKDSDDVPMVLVGNKCDLAARTVESRQAQDLARSYGIPYIETSAKTRQGVEDAFYTLVREIRQHKLRKLNPPDESGPGCMSCKCVLS

SEQ ID NO: 20 - protein, 189 aa, Homo sapiens
MTEYKLVVVGAGGVGKSALTIQLIQNHFVDEYDPTIEDSYRKQVVIDGETCLLDILDTAGQEEYSAMRDQYMRTGEGFLCVFAINNSKSFADINLYREQIKRVKDSDDVPMVLVGNKCDLPTRTVDTKQAHELAKSYGIPFIETSAKTRQGVEDAFYTLVREIRQYRMKKLNSSDDGTQGCMGLPCVVM

SEQ ID NO: 21 - protein, 189 aa, Homo sapiens
MTEYKLVVVGAVGVGKSALTIQLIQNHFVDEYDPTIEDSYRKQVVIDGETCLLDILDTAGQEEYSAMRDQYMRTGEGFLCVFAINNTKSFEDIHHYREQIKRVKDSEDVPMVLVGNKCDLPSRTVDTKQAQDLARSYGIPFIETSAKTRQRVEDAFYTLVREIRQYRLKKISKEEKTPGCVKIKKCIIM

SEQ ID NO: 22 - protein, 188 aa, Homo sapiens
MTEYKLVVVGAVGVGKSALTIQLIQNHFVDEYDPTIEDSYRKQVVIDGETCLLDILDTAGQEEYSAMRDQYMRTGEGFLCVFAINNTKSFEDIHHYREQIKRVKDSEDVPMVLVGNKCDLPSRTVDTKQAQDLARSYGIPFIETSAKTRQGVDDAFYTLVREIRKHKEKMSKDGKKKKKKSKTKCVIM

SEQ ID NO: 23 - protein, 189 aa, Homo sapiens [sequence omitted]

SEQ ID NO: 24 - protein, 189 aa, Homo sapiens
MTEYKLVVVGAVGVGKSALTIQLIQNHFVDEYDPTIEDSYRKQVVIDGETCLLDILDTAGQEEYSAMRDQYMRTGEGFLCVFAINNSKSFADINLYREQIKRVKDSDDVPMVLVGNKCDLPTRTVDTKQAHELAKSYGIPFIETSAKTRQGVEDAFYTLVREIRQYRMKKLNSSDDGTQGCMGLPCVVM

SEQ ID NO: 25 - protein, 189 aa, Homo sapiens
MTEYKLVVVGACGVGKSALTIQLIQNHFVDEYDPTIEDSYRKQVVIDGETCLLDILDTAGQEEYSAMRDQYMRTGEGFLCVFAINNTKSFEDIHHYREQIKRVKDSEDVPMVLVGNKCDLPSRTVDTKQAQDLARSYGIPFIETSAKTRQRVEDAFYTLVREIRQYRLKKISKEEKTPGCVKIKKCIIM

SEQ ID NO: 26 - protein, 188 aa, Homo sapiens
MTEYKLVVVGACGVGKSALTIQLIQNHFVDEYDPTIEDSYRKQVVIDGETCLLDILDTAGQEEYSAMRDQYMRTGEGFLCVFAINNTKSFEDIHHYREQIKRVKDSEDVPMVLVGNKCDLPSRTVDTKQAQDLARSYGIPFIETSAKTRQGVDDAFYTLVREIRKHKEKMSKDGKKKKKKSKTKCVIM

SEQ ID NO: 27 - protein, 189 aa, Homo sapiens
MTEYKLVVVGACGVGKSALTIQLIQNHFVDEYDPTIEDSYRKQVVIDGETCLLDILDTAGQEEYSAMRDQYMRTGEGFLCVFAINNTKSFEDIHQYREQIKRVKDSDDVPMVLVGNKCDLAARTVESRQAQDLARSYGIPYIETSAKTRQGVEDAFYTLVREIRQHKLRKLNPPDESGPGCMSCKCVLS

SEQ ID NO: 28 - protein, 189 aa, Homo sapiens
MTEYKLVVVGACGVGKSALTIQLIQNHFVDEYDPTIEDSYRKQVVIDGETCLLDILDTAGQEEYSAMRDQYMRTGEGFLCVFAINNSKSFADINLYREQIKRVKDSDDVPMVLVGNKCDLPTRTVDTKQAHELAKSYGIPFIETSAKTRQGVEDAFYTLVREIRQYRMKKLNSSDDGTQGCMGLPCVVM

SEQ ID NO: 29 - protein, 23 aa, Homo sapiens
TEYKLVVVGAGGVGKSALTIQLI

SEQ ID NO: 30 - protein, 137 aa, Artificial Sequence
  Synthetic
  MISC_FEATURE (48)..(48): X is Thr or Cys
  MISC_FEATURE (112)..(112): X is Ser, Ala, Val, Leu, Ile, Pro, Phe, Met, or Trp
  MISC_FEATURE (114)..(114): X is Met, Ala, Val, Leu, Ile, Pro, Phe, or Trp
  MISC_FEATURE (115)..(115): X is Gly, Ala, Val, Leu, Ile, Pro, Phe, Met, or Trp
DIQNPEPAVYQLKDPRSQDSTLCLFTDFDSQINVPKTMESGTFITDKXVLDMKAMDSKSNGAIAWSNQTSFTCQDIFKETNATYPSSDVPCDATLTEKSFETDMNLNFQNLXVXXLRILLLKVAGFNLLMTLRLWSS

SEQ ID NO: 31 - protein, 173 aa, Artificial Sequence
  Synthetic
  MISC_FEATURE (57)..(57): X is Ser or Cys
EDLRNVTPPKVSLFEPSKAEIANKQKATLVCLARGFFPDHVELSWWVNGKEVHSGVXTDPQAYKESNYSYCLSSRLRVSATFWHNPRNHFRCQVQFHGLSEEDKWPEGSPKPVTQNISAEAWGRADCGITSASYQQGVLSATILYEILLGKATLYAVLVSTLVVMAMVKRKNS

SEQ ID NO: 32 - protein, 137 aa, Mus musculus
DIQNPEPAVYQLKDPRSQDSTLCLFTDFDSQINVPKTMESGTFITDKTVLDMKAMDSKSNGAIAWSNQTSFTCQDIFKETNATYPSSDVPCDATLTEKSFETDMNLNFQNLSVMGLRILLLKVAGFNLLMTLRLWSS

SEQ ID NO: 33 - protein, 173 aa, Mus musculus
EDLRNVTPPKVSLFEPSKAEIANKQKATLVCLARGFFPDHVELSWWVNGKEVHSGVSTDPQAYKESNYSYCLSSRLRVSATFWHNPRNHFRCQVQFHGLSEEDKWPEGSPKPVTQNISAEAWGRADCGITSASYQQGVLSATILYEILLGKATLYAVLVSTLVVMAMVKRKNS

SEQ ID NO: 34 - protein, 268 aa, Artificial Sequence
  Synthetic
  MISC_FEATURE (179)..(179): X is Thr or Cys
  MISC_FEATURE (243)..(243): X is Ser, Ala, Val, Leu, Ile, Pro, Phe, Met, or Trp
  MISC_FEATURE (245)..(245): X is Met, Ala, Val, Leu, Ile, Pro, Phe, or Trp
  MISC_FEATURE (246)..(246): X is Gly, Ala, Val, Leu, Ile, Pro, Phe, Met, or Trp
MTSIRAVFIFLWLQLDLVNGENVEQHPSTLSVQEGDSAVIKCTYSDSASNYFPWYKQELGKGPQLIIDIRSNVGEKKDQRIAVTLNKTAKHFSLHITETQPEDSAVYFCAASTGGGNKLTFGTGTQLKVELDIQNPEPAVYQLKDPRSQDSTLCLFTDFDSQINVPKTMESGTFITDKXVLDMKAMDSKSNGAIAWSNQTSFTCQDIFKETNATYPSSDVPCDATLTEKSFETDMNLNFQNLXVXXLRILLLKVAGFNLLMTLRLWSS

SEQ ID NO: 35 - protein, 305 aa, Artificial Sequence
  Synthetic
  MISC_FEATURE (189)..(189): X is Ser or Cys
MLLLLLLLGPAGSGLGAVVSQHPSRVICKSGTSVKIECRSLDFQATTMFWYRQFPKQSLMLMATSNEGSKATYEQGVEKDKFLINHASLTLSTLTVTSAHPEDSSFYICSAREGAGGMGTQYFGPGTRLLVLEDLRNVTPPKVSLFEPSKAEIANKQKATLVCLARGFFPDHVELSWWVNGKEVHSGVXTDPQAYKESNYSYCLSSRLRVSATFWHNPRNHFRCQVQFHGLSEEDKWPEGSPKPVTQNISAEAWGRADCGITSASYQQGVLSATILYEILLGKATLYAVLVSTLVVMAMVKRKNS

SEQ ID NO: 36 - protein, 269 aa, Artificial Sequence
  Synthetic
  MISC_FEATURE (180)..(180): X is Thr or Cys
  MISC_FEATURE (244)..(244): X is Ser, Ala, Val, Leu, Ile, Pro, Phe, Met, or Trp
  MISC_FEATURE (246)..(246): X is Met, Ala, Val, Leu, Ile, Pro, Phe, or Trp
  MISC_FEATURE (247)..(247): X is Gly, Ala, Val, Leu, Ile, Pro, Phe, Met, or Trp
MEKNPLAAPLLILWFHLDCVSSILNVEQSPQSLHVQEGDSTNFTCSFPSSNFYALHWYRWETAKSPEALFVMTLNGDEKKKGRISATLNTKEGYSYLYIKGSQPEDSATYLCAFTTGNQFYFGTGTSLTVIPDIQNPEPAVYQLKDPRSQDSTLCLFTDFDSQINVPKTMESGTFITDKXVLDMKAMDSKSNGAIAWSNQTSFTCQDIFKETNATYPSSDVPCDATLTEKSFETDMNLNFQNLXVXXLRILLLKVAGFNLLMTLRLWSS

SEQ ID NO: 37 - protein, 310 aa, Artificial Sequence
  Synthetic
  MISC_FEATURE (194)..(194): X is Ser or Cys
MGSWTLCCVSLCILVAKHTDAGVIQSPRHEVTEMGQEVTLRCKPISGHDYLFWYRQTMMRGLELLIYFNNNVPIDDSGMPEDRFSAKMPNASFSTLKIQPSEPRDSAVYFCASSSYGGYSNQPQHFGDGTRLSILEDEDLRNVTPPKVSLFEPSKAEIANKQKATLVCLARGFFPDHVELSWWVNGKEVHSGVXTDPQAYKESNYSYCLSSRLRVSATFWHNPRNHFRCQVQFHGLSEEDKWPEGSPKPVTQNISAEAWGRADCGITSASYQQGVLSATILYEILLGKATLYAVLVSTLVVMAMVKRKNS

SEQ ID NO: 38 - protein, 268 aa, Artificial Sequence
  Synthetic
MTSIRAVFIFLWLQLDLVNGENVEQHPSTLSVQEGDSAVIKCTYSDSASNYFPWYKQELGKGPQLIIDIRSNVGEKKDQRIAVTLNKTAKHFSLHITETQPEDSAVYFCAASTGGGNKLTFGTGTQLKVELDIQNPEPAVYQLKDPRSQDSTLCLFTDFDSQINVPKTMESGTFITDKTVLDMKAMDSKSNGAIAWSNQTSFTCQDIFKETNATYPSSDVPCDATLTEKSFETDMNLNFQNLSVMGLRILLLKVAGFNLLMTLRLWSS

SEQ ID NO: 39 - protein, 305 aa, Artificial Sequence
  Synthetic
MLLLLLLLGPAGSGLGAVVSQHPSRVICKSGTSVKIECRSLDFQATTMFWYRQFPKQSLMLMATSNEGSKATYEQGVEKDKFLINHASLTLSTLTVTSAHPEDSSFYICSAREGAGGMGTQYFGPGTRLLVLEDLRNVTPPKVSLFEPSKAEIANKQKATLVCLARGFFPDHVELSWWVNGKEVHSGVSTDPQAYKESNYSYCLSSRLRVSATFWHNPRNHFRCQVQFHGLSEEDKWPEGSPKPVTQNISAEAWGRADCGITSASYQQGVLSATILYEILLGKATLYAVLVSTLVVMAMVKRKNS

SEQ ID NO: 40 - protein, 269 aa, Artificial Sequence
  Synthetic
MEKNPLAAPLLILWFHLDCVSSILNVEQSPQSLHVQEGDSTNFTCSFPSSNFYALHWYRWETAKSPEALFVMTLNGDEKKKGRISATLNTKEGYSYLYIKGSQPEDSATYLCAFTTGNQFYFGTGTSLTVIPDIQNPEPAVYQLKDPRSQDSTLCLFTDFDSQINVPKTMESGTFITDKTVLDMKAMDSKSNGAIAWSNQTSFTCQDIFKETNATYPSSDVPCDATLTEKSFETDMNLNFQNLSVMGLRILLLKVAGFNLLMTLRLWSS

SEQ ID NO: 41 - protein, 310 aa, Artificial Sequence
  Synthetic
MGSWTLCCVSLCILVAKHTDAGVIQSPRHEVTEMGQEVTLRCKPISGHDYLFWYRQTMMRGLELLIYFNNNVPIDDSGMPEDRFSAKMPNASFSTLKIQPSEPRDSAVYFCASSSYGGYSNQPQHFGDGTRLSILEDEDLRNVTPPKVSLFEPSKAEIANKQKATLVCLARGFFPDHVELSWWVNGKEVHSGVSTDPQAYKESNYSYCLSSRLRVSATFWHNPRNHFRCQVQFHGLSEEDKWPEGSPKPVTQNISAEAWGRADCGITSASYQQGVLSATILYEILLGKATLYAVLVSTLVVMAMVKRKNS

SEQ ID NO: 42 - DNA, 393 bp, Homo sapiens
atgaccagcatcagggccgtgttcatcttcctgtggctgcagctggacctggtgaacggcgagaacgtggagcagcaccccagcaccctgagcgtgcaggagggcgacagcgccgtgatcaagtgcacctacagcgacagcgccagcaactacttcccctggtacaagcaggagctgggcaagggcccccagctgatcatcgacatcaggagcaacgtgggcgagaagaaggaccagaggatcgccgtgaccctgaacaagaccgccaagcacttcagcctgcacatcaccgagacccagcccgaggacagcgccgtgtacttctgcgccgccagcaccggcggcggcaacaagctgaccttcggcaccggcacccagctgaaggtggagctg

SEQ ID NO: 43 - DNA, 393 bp, Homo sapiens; identical to SEQ ID NO: 42

SEQ ID NO: 44 - DNA, 396 bp, Homo sapiens
atggagaagaaccccctggccgcccccctgctgatcctgtggttccacctggactgcgtgagcagcatcctgaacgtggagcagagcccccagagcctgcacgtgcaggagggcgacagcaccaacttcacctgcagcttccccagcagcaacttctacgccctgcactggtacaggtgggagaccgccaagagccccgaggccctgttcgtgatgaccctgaacggcgacgagaagaagaagggcaggatcagcgccaccctgaacaccaaggagggctacagctacctgtacatcaagggcagccagcccgaggacagcgccacctacctgtgcgccttcaccaccggcaaccagttctacttcggcaccggcaccagcctgaccgtgatcccc

SEQ ID NO: 45 - DNA, 411 bp, Homo sapiens
atgggcagctggaccctgtgctgcgtgagcctgtgcatcctggtggccaagcacaccgacgccggcgtgatccagagccccaggcacgaggtgaccgagatgggccaggaggtgaccctgaggtgcaagcccatcagcggccacgactacctgttctggtacaggcagaccatgatgaggggcctggagctgctgatctacttcaacaacaacgtgcccatcgacgacagcggcatgcccgaggacaggttcagcgccaagatgcccaacgccagcttcagcaccctgaagatccagcccagcgagcccagggacagcgccgtgtacttctgcgccagcagcagctacggcggctacagcaaccagccccagcacttcggcgacggcaccaggctgagcatcctggaggac

SEQ ID NO: 46 - protein, 11 aa, Homo sapiens
LVVVGAVGVGK

SEQ ID NO: 47 - protein, 12 aa, Homo sapiens
KLVVVGAVGVGK

SEQ ID NO: 48 - protein, 12 aa, Homo sapiens
LVVVGAVGVGKS

SEQ ID NO: 49 - protein, 13 aa, Homo sapiens
YKLVVVGAVGVGK

SEQ ID NO: 50 - protein, 13 aa, Homo sapiens
KLVVVGAVGVGKS

SEQ ID NO: 51 - protein, 13 aa, Homo sapiens
LVVVGAVGVGKSA

SEQ ID NO: 52 - protein, 15 aa, Homo sapiens
EYKLVVVGAVGVGKS

SEQ ID NO: 53 - protein, 24 aa, Homo sapiens
MTEYKLVVVGAVGVGKSALTIQLI

SEQ ID NO: 54 - protein, 27 aa, Artificial Sequence
  Synthetic
RAKRSGSGATNFSLLKQAGDVEENPGP

SEQ ID NO: 55 - protein, 24 aa, Homo sapiens
MTEYKLVVVGAGGVGKSALTIQLI

SEQ ID NO: 56 - protein, 24 aa, Homo sapiens
MTEYKLVVVGACGVGKSALTIQLI